European Patent Application EP 4 534 679 A2, published April 9, 2025. Title: A method for improving the mean dry shoot weight, mean dry grain weight, and suppressing seed-borne infection in a cereal crop. Applicant: The Provost, Fellows, Scholars and other Members of Board of Trinity College Dublin. Application EP. The sequence listing filed with the application follows.

SEQUENCE LISTING (15 sequences)

SEQ ID NO: 1 - DNA, 19 bp, synthetic construct
  misc_feature 1..19: note = Forward Primer
  source 1..19: mol_type = other DNA
tccgtaggtgaacctgcgg

SEQ ID NO: 2 - DNA, 20 bp, synthetic construct
  misc_feature 1..20: note = Reverse Primer
  source 1..20: mol_type = other DNA
tcctccgcttattgatatgc

SEQ ID NO: 3 - DNA, 671 bp, unidentified
  misc_feature 1..671: note = nuclear ribosomal internal transcribed spacer (nrITS) sequence
  source 1..671: mol_type = genomic DNA
gcctaagctcccaaaacccactgtgacatatacctttgttttcgttgcctcggcggggtcgtgctccctggaaacaggggttcgcgccgccgggtgacacctaaaccctgatttaattacagaagtctttctgagtaaaacattctaaatgaatcaaaactttcaacaacggatctcttggttctggcatcgatgaagaacgcagcgaaatgcgataagtaatgtgaattgcagaattcagtgaatcatcgaatctttgaacgcacattgcgcccgccagtattctggcgggcatgcctgttcgagcgtcatttcaaccctcaagaccccttcgggggacttggtgttggggaccggctgttcccggcctgcttcttgcagcgcctttatgccgcccccgaaatgaattggcggcctcgtcgcggcctcccctgcgtagtagcacaacctcgcaacgggaacgtgacggcggccctgccgtaaacaacccaattttattaaagttgacctcgaatcagggaggatacccgctgaacttaagcatatcataaggggaggaaagaccgacgaaattgcccattaaccgcagggatcgcctcgctcaattcgaatcagccctagcccgactcctcggtaccctaagaaatcccaatttccccctttttttacat

SEQ ID NO: 4 - DNA, 656 bp, unidentified
  misc_feature 1..656: note = nuclear ribosomal internal transcribed spacer (nrITS) sequence
  source 1..656: mol_type = genomic DNA
ttagaaggcgtctccttttgacaaaacccaccccgtgtatcttctgagggggccctgtgatattcccctcgcggggcaggagggccgttctacgaatcctcggtcggtggcctgctggggaggccggggcccgctgggggggcctctgccagccgcctgggacttgcgtcccgggggtgctggcgccgaccgccaggatccctgtaccaaactattgagatttgaaatatgacaaaatcaaaccattacaacctgcaacgatggatctcttggctctggcatcgatgaagaacgcagcgaaatgcgatacgtaatgtgaattgcagatctctcagtgaatcatcgagtttttgaacgcacatagcgcccgccagcattctggcgggcatggcctgtccgagcgtcgatgacgcctgctcgagcgctgccgctcggtgttggggcgctaggggcctcgccccctaggccctctaagaagaagtgcgcggtccacgacgggccccgggtacagtaatttattgctgccctagggagccgccgggcgggcttggccgtaaaacccccgacataggccgagccctgctgcagggtgaccccgccatatgttgacctcggatccaggtaggacgacccgctgaacttaagcatatcaatag

SEQ ID NO: 5 - DNA, 520 bp, unidentified
  misc_feature 1..520: note = nuclear ribosomal internal transcribed spacer (nrITS) sequence
  source 1..520: mol_type = genomic DNA
acctaagggatttcgggtcgggatgttcataaccctttgttgtccgactctgttgcctccggggcgaccctgccttcgggcgggggctccgggtggacacttcaaactcttgcgtaactttgcagtctgagtaaacttaattaataaattaaaacttttaacaacggatctcttggttctggcatcgatgaagaacgcagcgaaatgcgataagtaatgtgaattgcagaattcagtgaatcatcgaatctttgaacgcacattgcgccccctggtattccggggggcatgcctgttcgagcgtcatttcaccactcaagcctcgcttggtattgggcaacgcggtccgccgcgtgcctcaaatcgtccggctgggtcttctgtccctaagcgttgtggaaactattcgctaaagggtgttcgggaggctacgccgtaaaaacaaccccatttctaaggttgacctcggatcaggtagggatacccgctgaacttaagcatatcataacgcgggagaaaa

SEQ ID NO: 6 - DNA, 573 bp, unidentified
  misc_feature 1..573: note = nuclear ribosomal internal transcribed spacer (nrITS) sequence
  source 1..573: mol_type = genomic DNA
ggggggttcctttcaaccctccggtgcggtttaatcttgtaacgcgtctgaatctggctgtcgtgcgtatcttgttccttctctgcttgtctgatatgatatctgtccgcgtctccgcgctcgccgaagacaccttagaactctgtctgaagattgtagtctgagattaaatataaattatttaaaactttcaacaacggatctcttggttccggcatcgatgaagaacgcaccgaaatgcgatacgtaatgtgaattgcagaattcagtgaatcatcgagtctttgaacgcacattgcgccctctggtattccggagggcatgctgtccgagcgtcattgctgcctcaagcacggttgtgtgtgggctccgtcctccttccggggacgggcccgaaggcgcgcggccccgccggcctcagcgatggggttgcaccgtttgagatggcgggctgcgtcacaattttcaggtgctcgacggaggtaccgtgactagcttcataagaagaaagaacaccgatgccatacgggtgaggcaaacaaattaacggtctcgtcccagtcactcaaaatt

SEQ ID NO: 7 - DNA, 521 bp, unidentified
  misc_feature 1..521: note = nuclear ribosomal internal transcribed spacer (nrITS) sequence
  source 1..521: mol_type = genomic DNA
gcatccatggatagcacttcactgttgcctgtctgacccttgtcttttgcgtactatttgtttcctcggtgggcttgcctgccgataggacaaccattaaaccttttgtaattgcaatcagcgtcagaaaaaacataatagttacaactttcaacaacggatctcttggttctggcatcgatgaagaacgcagcgaaatgcgaaaagtagtgtgaattgcagaattcagtgaatcatcgaatctttgaacgcacattgcgccccttggtattccatggggcatgcctgttcgagcgtcatttgtaccttcaagccctgcttggtgttgggtgtttgtcccgctttgtgcgtggactcgcctcaaagcaattggcagccggcgtactagcctgggagcgcagcacattttgcgcatcttgtcttgaacgcttgcgtccatgaagcctacattttaactcttgacctcggatcaggtagggatacccgctgaacttaagcatatcaaaggggggggagaaaaa

SEQ ID NO: 8 - DNA, 757 bp, unidentified
  misc_feature 1..757: note = nuclear ribosomal internal transcribed spacer (nrITS) sequence
  source 1..757: mol_type = genomic DNA
tagaaaaccaacccctgtgattatacctttaattgttgcttcggcgggacttcgcgcccgccggggacccaaaccttctgaattttttaataagtatcttctgagtggttaaaaaaatgaatcaaaactttcaacaacggatctcttggttctggcatcgatgaagaacgcagcgaaatgcgataagtaatgtgaattgcagaattcagtgaatcatcgaatctttgaacgcacattgcgcccgtcagtattctggcgggcatgcctgttcgagcgtcattacgcccctcaagtcccctgtgggacttggtgttggggatcggcgaggcttggttttccagcgcagccgtccctcaaatcaattggcgggtctcgcccgtggccctccctctgcgcagtagtaaaaaccacctccgcaacaggagcccggcgccgttcccactgcccgtaaaaacccccccaacttttttatagttgacctccggaatcagggtaaggactaccccgcctgaaacttaaagcatatctaaagcggggggagagagaaaacccccccccgggggggggtgggggcaaacccacccgcaaaaattttaggccggggcaatctccccccctgtggggggggccctccaaccccttaagcgccaatcgaacctgggttacgttgatcccgccaacccccgggcccgggggggaattccccgcctgaaattttaaagctttatcatataagggggagagagaaagggggaaa

SEQ ID NO: 9 - DNA, 517 bp, unidentified
  misc_feature 1..517: note = nuclear ribosomal internal transcribed spacer (nrITS) sequence
  source 1..517: mol_type = genomic DNA
ccctcactatttcttatttgcagagtatgccgcggtcaggcttcccctgccaggagtgagtctggcagcacatcctcattgcaactacgagagcggtcccgcctacggcagctacttatcgacacgagctgttgactagtgcctactaatgttcctcgttgaagggcaataattgctatgctcgttggccaaaacgccgaggtgccataaaattggcagaactcttgggattcagagggactttgaccggtaatggctttccccaggttcccctaccaaaaacttctctgagccttcgtgatgtccacaagctacgttggtgagtagggttccgccttctctcctgggggaagggcaagaaaggcagcggcggtaccgcgtccggtcctcaagcgtatggggctttgtcacccgctttgtaggatggccggcgccgccgatcaaccaaactttttccaggttgacctcggatcaggtagggttacccgctgaacttagcatatcataagcggagaaa

SEQ ID NO: 10 - DNA, 581 bp, unidentified
  misc_feature 1..581: note = nuclear ribosomal internal transcribed spacer (nrITS) sequence
  source 1..581: mol_type = genomic DNA
acttaagaaggatgtcgagagcctaacctattccacactgaagattcgatccctagtgcctgcaggagatgcctaccggggcagaacttcgaaggtcttaatccaagatgtctttgtctgagtgttctcttttaaatccagctaatctttcaacaacggatctcttggttctggcatcgatgaagaacgcagcgaaatgcgataagtaatgcgaattgcagaattctcgtgagtcatcgaatctttgaacgcacattgcgccctttggtattccgaagggcatgcctgttcgagcgtcattttcacccctcaagcccccggcttggtgttggacggtctggtccggggacctcaaaccccctggacccctcccaaagacaatgacggcgggctgttgaacccccggtacactggagcatcttcacggagcacgtaccggtctcaagggtcgacggcacccggtctatacctatatttttcaaggttgacctcggatcaggtaggaatacccgctgaacttaagcatatcatagggggggagaaaagtcataaatgcaccagattctggtcactggggcggg

SEQ ID NO: 11 - DNA, 642 bp, unidentified
  misc_feature 1..642: note = nuclear ribosomal internal transcribed spacer (nrITS) sequence
  source 1..642: mol_type = genomic DNA
ttcccccacccccgtgttttattttaccttgttgcttcggcgagcctgccttttggctgccgggggacatctgtccccgggtccgcgctcgccgaagacaccttagaactctgtctgaagattgtagtctgagattaaatataaattatttaaaactttcaacaacggatctcttggttccggcatcgatgaagaacgcagcgaaatgcgatacgtaatgtgaattgcagaattcagtgaatcatcgagtctttgaacgcacattgcgccctctggtattccggagggcatgcctgtccgagcgtcattgctgccctcaagcacggcttgtgtgttgggctccgtcctccttccgggggacgggcccgaaaggcagcggcggcaccgcgtccggtcctcaagcgtatggggctttgtcaccccgctttgtaggactggccggcgcctgccgatcaaccaaacttttttccaggttgacctcggatcaggtaggggatacccgctgaacttaagcatatcataggcgggaggaaaggagctacggggattgccccagtaacggcgagtgaagcgcaagagctcagattctcagcgctccatccggtcccgcaagttcacctacagaaacgggagtaaaaacct

SEQ ID NO: 12 - DNA, 628 bp, unidentified
  misc_feature 1..628: note = nuclear ribosomal internal transcribed spacer (nrITS) sequence
  source 1..628: mol_type = genomic DNA
cggtttattttaaccttgttgcttcggcgagccttgccttttggctgccgggggacatctgtccccgggtccgcgctcgccgaagacaccttagaactctgtctgaagattgtagtctgagattaaatataaattatttaaaactttcaacaacggatctcttggttccggcatcgatgaagaacgcagcgaaatgcgatacgtaatgtgaattgcagaattcagtgaatcatcgagtctttgaacgcacattgcgccctctggtattccggagggcatgcctgtccgagcgtcattgctgccctcaagcacggcttgtgtgttgggctccgtcctccttccgggggacgggcccgaaaggcagcggcggcaccgcgtccggtcctcaagcgtatggggctttgtcaccccgctttgtaggactggccggcgcctgccgatcaaccaaacttttttccaggttgacctcggatcaggtagggatacccgctgaacttaagcatatcataagcgcggaagggaaacagaacctacgggagattgccccataacagcgagtgaagcgcaagagctcaatttgtaagtcggctcctcgggtcccccagtcacactacgaaaaggcctgatt

SEQ ID NO: 13 - DNA, 793 bp, unidentified
  misc_feature 1..793: note = nuclear ribosomal internal transcribed spacer (nrITS) sequence
  source 1..793: mol_type = genomic DNA
tttggatttttaccggcgtagcctcccgaacaccctttagcgaatagtttccacaacgcttaggggacagaagtacccagccggacgaattttgaaggcacgcggcggaaccgcgtttgcccaataccaagcgaggctttgagtgggtgaaaatgaacgccttcgaaacagggcatggccccccccgggaaataaccagggggggccgccaatggtgccgtttcaaaggaatttcgattgaatttcactggaaatttctggcaaatttcacatttaacttattcgcatttttcgctgccgtttctttcattcgattgcccagaaaccaaagaggaatccgttggttaaaaggttttaattttaattaaattaaagtttaacttcagaactgcaaaggttaacgccaagagttttgaaggtggtcccaccccgggtgccccccgccccgaagggcaggggttcgccccccggaggcaaacagagtccggaacaaacaaaaggggttaatgaaacattccccgggcccgttagcccgggggttcactttgtaattgattccctttcgagtcccccccccccaaaaaaaaaaaaccccgggggggcccccgggaaaagcggggatttttttttaaaccccttttttttccggactctttttgccccccggggggaaccctgtgttttttggggcggggccctccgggtgggaccccttcaaaactcgtgctaaaacttttcgggctgggggtaaactttatttaaaaaattaaaaacttttttaaaaaacggggac

SEQ ID NO: 14 - DNA, 716 bp, unidentified
  misc_feature 1..716: note = nuclear ribosomal internal transcribed spacer (nrITS) sequence
  source 1..716: mol_type = genomic DNA
ccctgcggggtgtacaaagccccatacgctcgaggaccggactcggtgccgccgctgcctttcggacccgtccccggggggacggagcccaacacacaagccgtgcttgaagggcagcaatgacgcttcggaacaggcatgccccccccgggaaataaccaggggggcggcaatggtgccgtttcaaaagaactccgattgaatttcacttgaaatttttgcaaatttcaacattaagttaatcggcattttcgctgccgttctttcatcgaatgcccgggaaaccaaagaaaatccgttgtttgaaaggttttaaacttaatttaggtttaatgcttcagaatggcaatctttcagaacagagttcaataagtgtcctccggtgcgccgcggaacccgggggcagaaagccccccccggccggcccgtgatgggcggggcgcacccgatgcaaccatggtacaattaaaacacgggtggggagtggttgggaccccagatgggcccttcactcagtaatgatcctatcggtcttttttagaaaaaaaaaaagaagcttttttacaacccccccccctttttcacaaaaccccccccccgtttttttctgcacactcttttgtctagggcggcggcttagccccacagaggggtctttctgcccccgggtccgcgcgccccggggaaaaaacatttaaaactcttttttaaaaaag

SEQ ID NO: 15 - DNA, 772 bp, unidentified
  misc_feature 1..772: note = nuclear ribosomal internal transcribed spacer (nrITS) sequence
  source 1..772: mol_type = genomic DNA
tcggggatcaaagcatatcaaatgttgcttactggatgccacccgccgcgacgagagacgcaattctgctgcgctcaaaagccgcttggtgtgggcttgccaatccgttttataggcgaagtcccgcgccgatgcgggacaagaacgcccaacaccaaagcttgtgctttgagggggtgtaaatggaccggcctccgaacaaggcatgcccctaaaggaaataccaaaaggggcggcaatggtggcgtttcaagagattcgaatgaattcactgaaatttctgccaatttcacactaactttattcgcatttttgcctgccgtttctttcattcgaatgcccagaaacccaagaagaatcccatttgtttgaaaagtttttgattcttctgtctgtccctcagaacgatttactggtattttacaaagaagtttgagggggtcccccagtagccaggccaagccttgctgaggaaacgaacgggtgctccaaaaaattaggcatggacgctatcctcgaccaggacaaaagcccttacgataatgatccttccgcagcccccgaagagagagtctttggggggtttttgtcccgtgaaaaaagcgcccctatgccttattttggggagcaccgttgttttcctcgggagggcttgcccgcatactggggaacccccacacacttttggtaaaatacagattatcgctctggaaacaaaccaaaatccaaatctctcaacaatgaaacctctgtgtttgcgcctcaataaaaa